European Patent Application EP 4 428 156 A1, published September 11, 2024. Title: ANTI-BCMA NANOBODY AND USE THEREOF. Applicant: Jiangsu Simcere Pharmaceutical Co., Ltd. The sequence listing filed with the application follows.

SEQUENCE LISTING (157 sequences)

SEQ ID NO: 1 - protein, 125 aa, Artificial sequence
EVQLVESGGGLVQPGGSLRLSCAASGFTFSNFWMTWVRQAPGKGLEWVANMNQDGSEKYYVDSVKGRFTISRDNAKSSLYLQMNSLRAEDTAVYYCARDREYCISTSCYDDFDYWGQGTLVTVSS

SEQ ID NO: 2 - protein, 108 aa, Artificial Sequence
DIQMTQSPSSLSASVGDRVTITCRASQSISSYLNWYQQKPGKAPKLLIYAASSLQSGVPSRFSGSGSGTDFTLTISSLQPEDFATYYCQQSYSTPPITFGQGTRLEIK

SEQ ID NO: 3 - protein, 119 aa, Artificial sequence
EVQLVESGGGLVQPGRSLTLSCAASTNIFSISPYGWYRQAPGKQRELVAAIHGTSTLYADSVKGRFTISRDNAKNSIYLQMNSLRPEDTALYYCNKVPWGDYHPGNVYWGQGTQVTVSS

SEQ ID NO: 4 - protein, 232 aa, Artificial Sequence
EPKSSDKTHTCPPCPAPELLGGPSVFLFPPKPKDTLMISRTPEVTCVVVDVSHEDPEVKFNWYVDGVEVHNAKTKPREEQYNSTYRVVSVLTVLHQDWLNGKEYKCKVSNKALPAPIEKTISKAKGQPREPQVYTLPPSREEMTKNQVSLTCLVKGFYPSDIAVEWESNGQPENNYKTTPPVLDSDGSFFLYSKLTVDKSRWQQGNVFSCSVMHEALHNHYTQKSLSLSPGK

SEQ ID NO: 5 - protein, 330 aa, Artificial Sequence
ASTKGPSVFPLAPSSKSTSGGTAALGCLVKDYFPEPVTVSWNSGALTSGVHTFPAVLQSSGLYSLSSVVTVPSSSLGTQTYICNVNHKPSNTKVDKKVEPKSCDKTHTCPPCPAPELLGGPSVFLFPPKPKDTLMISRTPEVTCVVVDVSHEDPEVKFNWYVDGVEVHNAKTKPREEQYNSTYRVVSVLTVLHQDWLNGKEYKCKVSNKALPAPIEKTISKAKGQPREPQVYTLPPSREEMTKNQVSLTCLVKGFYPSDIAVEWESNGQPENNYKTTPPVLDSDGSFFLYSKLTVDKSRWQQGNVFSCSVMHEALHNHYTQKSLSLSPGK

SEQ ID NO: 6 - protein, 107 aa, Artificial Sequence [sequence omitted]

SEQ ID NO: 7 - protein, 126 aa, Artificial Sequence
QVQLVESGGGLVQPGGSLRLSCSGSGFTLDYYMIGWFRQAPGKEREGLSSISPADGSTYYADSVKGRFTISRDSAKNTVYLQMNNLKPEDTALYYCAAGNEATISWGFGPWEYDYWGQGTQVTVSS

SEQ ID NO: 8 - protein, 123 aa, Artificial Sequence
QVQLVESGGGLVQSRGSLRLSCAASESISSIHIMAWYRRAPGKQRELVAGIRNDGSTVYADSAKGRFTISRDNAKNTVYLQMNSLKPEDTAVYYCNADQGFGSYSEWERRSRWGQGTEVTVSS

SEQ ID NO: 9 - protein, 126 aa, Artificial Sequence
EVQVVESGGGLVQPGGSLRLSCAGSGFTLAHYMIGWFRQAPGKEREGLSSISPADGSTYYADSVKGRFTISRDNAKNTVYLQMNSLKPEDTALYYCAAGNEATISWGFGPYEYDYWGQGTQVTVSS

SEQ ID NO: 10 - protein, 126 aa, Artificial Sequence
EVQVVESGGGLVQPGGSLRLSCAGSGFTLAYYMIGWFRQAPGKEREGLSSISPADGSTYYADSVKGRFTISRDNAKNTVYLQMNSLKPEDTALYYCAAGNEAAITWGFGPYEYDYWGQGTQVTVSS

SEQ ID NO: 11 - protein, 126 aa, Artificial Sequence
QVQLVESGGGLVQPGGSLRLSCAASGFTLAYYMIGWFRQAPGKEREGVSSISSGTGSTYYANSVKDRFTISRDNAANKVYLEMNSLKPEDTAIYYCAAGNEATITWGFGPYEYDYWGQGTQVTVSS

SEQ ID NO: 12 - protein, 126 aa, Artificial Sequence
EVQVVESGGGLVQPGGSLRLSCAASGFTLAYYGIGWFRQAPGQEREGVASITASDGSTYYADSVKDRFTISRDNAANTVYLQMNSLKPEDTAVYFCAAGNDGAISWGFGPYEYDYWGQGTQVTVSS

SEQ ID NO: 13 - protein, 116 aa, Artificial Sequence
QVQLVESGGGLVQPGGSLRLSCAASGFTFRSSAMSWARQAPGKGLEWVSAIYPDGRTYYADSIKGRFTSSRDNAKNTVYLQMNSLRSEDTAIYYCTIGNQLSDLPLGQGTQVTVSS

SEQ ID NO: 14 - protein, 126 aa, Artificial Sequence
QVQLVESGGGLVQPGGSLRLSCTDSGFTLNYYMIGWFRQAPGKEQEGLSSISAGDGSTYYADSVKGRFTISRDYAKNTVYLEMNDLKPEDTGVYYCAAGNEGAITWGFGPYEYDYWGQGTQVTVSS

SEQ ID NO: 15 - protein, 126 aa, Artificial Sequence
EVQLVESGGGLVQPGGSLRLSCSASGFTLDYYMMGWFRQAPGKEREGVSSISPADGSTYYADSVKGRFTISRDNSKNTLYLQMNSLRAEDTAVYYCAAGNEATISWGFGPWEYDYWGQGTMVTVSS

SEQ ID NO: 16 - protein, 126 aa, Artificial Sequence
EVQLVESGGGLVQPGGSLRLSCSASGFTLDYYMMGWFRQAPGKEREGVSSISPADGSTYYADSVKGRFTISRDSSKNTLYLQMNSLRAEDTAVYYCAAGNEATISWGFGPWEYDYWGQGTMVTVSS

SEQ ID NO: 17 - protein, 126 aa, Artificial sequence
EVQLVESGGGLVQPGGSLRLSCSASGFTLDYYMIGWFRQAPGKEREGVSSISPADGSTYYADSVKGRFTISRDSSKNTVYLQMNSLRAEDTAVYYCAAGNEATISWGFGPWEYDYWGQGTMVTVSS

SEQ ID NO: 18 - protein, 126 aa, Artificial Sequence
EVQLVESGGGLVQPGGSLRLSCSASGFTLDYYMIGWFRQAPGKEREGVSSISPADGSTYYADSVKGRFTISRDSAKNTVYLQMNSLRAEDTAVYYCAAGNEATISWGFGPWEYDYWGQGTMVTVSS

SEQ ID NO: 19 - protein, 126 aa, Artificial Sequence
EVQLVESGGGLVQPGGSLRLSCSASGFTLDYYMIGWFRQAPGKEREGVSSISPADGSTYYADSVKGRFTISRDSSKNTVYLQMNSLRAEDTALYYCAAGNEATISWGFGPWEYDYWGQGTQVTVSS

SEQ ID NO: 20 - protein, 126 aa, Artificial Sequence
EVQLVESGGGLVQPGGSLRLSCSASGFTLDYYMIGWFRQAPGKEREGLSSISPADGSTYYADSVKGRFTISRDSSKNTVYLQMNSLRAEDTAVYYCAAGNEATISWGFGPWEYDYWGQGTMVTVSS

SEQ ID NO: 21 - protein, 126 aa, Artificial Sequence
QVQLVESGGGLVQPGGSLRLSCSASGFTLDYYMIGWFRQAPGKEREGVSSISPADGSTYYADSVKGRFTISRDSSKNTVYLQMNSLRAEDTAVYYCAAGNEATISWGFGPWEYDYWGQGTMVTVSS

SEQ ID NO: 22 - protein, 98 aa, Artificial Sequence
QVQLVESGGGLVQPGGSLRLSCSASGFTFSSYAMHWVRQAPGKGLEYVSAISSNGGSTYYADSVKGRFTISRDNSKNTLYLQMNSLRAEDTAVYYCAR

SEQ ID NO: 23 - protein, 11 aa, Artificial sequence
WGQGTMVTVSS

SEQ ID NO: 24 - protein, 123 aa, Artificial Sequence
EVQLVESGGGLVQPGGSLRLSCAASESISSIHIMSWYRQAPGKQRELVANIRNDGSTYYVDSVKGRFTISRDNAKNSLYLQMNSLRAEDTAVYYCNADQGFGSYSEWERRSRWGQGTTVTVSS

SEQ ID NO: 25 - protein, 123 aa, Artificial Sequence
EVQLVESGGGLVQPGGSLRLSCAASESISSIHIMAWYRQAPGKQRELVANIRNDGSTYYVDSVKGRFTISRDNAKNSLYLQMNSLRAEDTAVYYCNADQGFGSYSEWERRSRWGQGTTVTVSS

SEQ ID NO: 26 - protein, 123 aa, Artificial Sequence
EVQLVESGGGLVQPGGSLRLSCAASESISSIHIMAWYRQAPGKQRELVAGIRNDGSTYYVDSVKGRFTISRDNAKNSLYLQMNSLRAEDTAVYYCNADQGFGSYSEWERRSRWGQGTTVTVSS

SEQ ID NO: 27 - protein, 123 aa, Artificial Sequence
EVQLVESGGGLVQPGGSLRLSCAASESISSIHIMAWYRQAPGKQRELVAGIRNDGSTVYVDSVKGRFTISRDNAKNSLYLQMNSLRAEDTAVYYCNADQGFGSYSEWERRSRWGQGTTVTVSS

SEQ ID NO: 28 - protein, 123 aa, Artificial Sequence
EVQLVESGGGLVQPGGSLRLSCAASESISSIHIMAWYRRAPGKQRELVAGIRNDGSTVYVDSVKGRFTISRDNAKNSLYLQMNSLRAEDTAVYYCNADQGFGSYSEWERRSRWGQGTTVTVSS

SEQ ID NO: 29 - protein, 123 aa, Artificial Sequence
EVQLVESGGGLVQPGGSLRLSCAASESISSIHIMAWYRQAPGKQRELVAGIRNDGSTVYADSVKGRFTISRDNAKNSLYLQMNSLRAEDTAVYYCNADQGFGSYSEWERRSRWGQGTTVTVSS

SEQ ID NO: 30 - protein, 123 aa, Artificial Sequence
EVQLVESGGGLVQPGGSLRLSCAASESISSIHIMAWYRQAPGKQRELVAGIRNDGSTVYVDSVKGRFTISRDNAKNSVYLQMNSLRAEDTAVYYCNADQGFGSYSEWERRSRWGQGTTVTVSS

SEQ ID NO: 31 - protein, 123 aa, Artificial Sequence
EVQLVESGGGLVQPGGSLRLSCAASESISSIHIMAWYRRAPGKQRELVAGIRNDGSTVYVDSVKGRFTISRDNAKNSLYLQMNSLRAEDTAVYYCNADQGFGSYSEWERRSRWGQGTEVTVSS

SEQ ID NO: 32 - protein, 98 aa, Artificial Sequence
EVQLVESGGGLVQPGGSLRLSCAASGFTFSSYWMSWVRQAPGKGLEWVANIKQDGSEKYYVDSVKGRFTISRDNAKNSLYLQMNSLRAEDTAVYYCAR

SEQ ID NO: 33 - protein, 11 aa, Artificial Sequence
WGQGTTVTVSS

SEQ ID NO: 34 - protein, 5 aa, Artificial Sequence
YYMIG

SEQ ID NO: 35 - protein, 17 aa, Artificial Sequence
SISPADGSTYYADSVKG

SEQ ID NO: 36 - protein, 17 aa, Artificial Sequence
GNEATISWGFGPWEYDY

SEQ ID NO: 37 - protein, 8 aa, Artificial Sequence
GFTLDYYM

SEQ ID NO: 38 - protein, 8 aa, Artificial Sequence
ISPADGST

SEQ ID NO: 39 - protein, 19 aa, Artificial Sequence
AAGNEATISWGFGPWEYDY

SEQ ID NO: 40 - protein, 7 aa, Artificial Sequence
GFTLDYY

SEQ ID NO: 41 - protein, 6 aa, Artificial Sequence
SPADGS

SEQ ID NO: 42 - protein, 5 aa, Artificial Sequence
IHIMA

SEQ ID NO: 43 - protein, 16 aa, Artificial Sequence
GIRNDGSTVYADSAKG

SEQ ID NO: 44 - protein, 15 aa, Artificial Sequence
DQGFGSYSEWERRSR

SEQ ID NO: 45 - protein, 8 aa, Artificial Sequence
ESISSIHI

SEQ ID NO: 46 - protein, 7 aa, Artificial Sequence
IRNDGST

SEQ ID NO: 47 - protein, 17 aa, Artificial Sequence
NADQGFGSYSEWERRSR

SEQ ID NO: 48 - protein, 7 aa, Artificial Sequence
ESISSIH

SEQ ID NO: 49 - protein, 5 aa, Artificial Sequence
RNDGS

SEQ ID NO: 50 - protein, 5 aa, Artificial Sequence
HYMIG

SEQ ID NO: 51 - protein, 17 aa, Artificial Sequence
GNEATISWGFGPYEYDY

SEQ ID NO: 52 - protein, 8 aa, Artificial Sequence
GFTLAHYM

SEQ ID NO: 53 - protein, 19 aa, Artificial Sequence
AAGNEATISWGFGPYEYDY

SEQ ID NO: 54 - protein, 7 aa, Artificial Sequence
GFTLAHY

SEQ ID NO: 55 - protein, 17 aa, Artificial Sequence
GNEAAITWGFGPYEYDY

SEQ ID NO: 56 - protein, 8 aa, Artificial Sequence
GFTLAYYM

SEQ ID NO: 57 - protein, 19 aa, Artificial Sequence
AAGNEAAITWGFGPYEYDY

SEQ ID NO: 58 - protein, 7 aa, Artificial Sequence
GFTLAYY

SEQ ID NO: 59 - protein, 17 aa, Artificial Sequence
SISSGTGSTYYANSVKD

SEQ ID NO: 60 - protein, 17 aa, Artificial Sequence
GNEATITWGFGPYEYDY

SEQ ID NO: 61 - protein, 8 aa, Artificial Sequence
ISSGTGST

SEQ ID NO: 62 - protein, 19 aa, Artificial Sequence
AAGNEATITWGFGPYEYDY

SEQ ID NO: 63 - protein, 6 aa, Artificial Sequence
SSGTGS

SEQ ID NO: 64 - protein, 5 aa, Artificial Sequence
YYGIG

SEQ ID NO: 65 - protein, 17 aa, Artificial Sequence
SITASDGSTYYADSVKD

SEQ ID NO: 66 - protein, 17 aa, Artificial Sequence
GNDGAISWGFGPYEYDY

SEQ ID NO: 67 - protein, 8 aa, Artificial Sequence
GFTLAYYG

SEQ ID NO: 68 - protein, 8 aa, Artificial Sequence
ITASDGST

SEQ ID NO: 69 - protein, 19 aa, Artificial Sequence
AAGNDGAISWGFGPYEYDY

SEQ ID NO: 70 - protein, 6 aa, Artificial Sequence
TASDGS

SEQ ID NO: 71 - protein, 5 aa, Artificial Sequence
SSAMS

SEQ ID NO: 72 - protein, 16 aa, Artificial Sequence
AIYPDGRTYYADSIKG

SEQ ID NO: 73 - protein, 8 aa, Artificial Sequence
GNQLSDLP

SEQ ID NO: 74 - protein, 8 aa, Artificial Sequence
GFTFRSSA

SEQ ID NO: 75 - protein, 7 aa, Artificial Sequence
IYPDGRT

SEQ ID NO: 76 - protein, 10 aa, Artificial Sequence
TIGNQLSDLP

SEQ ID NO: 77 - protein, 7 aa, Artificial Sequence
GFTFRSS

SEQ ID NO: 78 - protein, 5 aa, Artificial Sequence
YPDGR

SEQ ID NO: 79 - protein, 17 aa, Artificial Sequence
SISAGDGSTYYADSVKG

SEQ ID NO: 80 - protein, 17 aa, Artificial Sequence
GNEGAITWGFGPYEYDY

SEQ ID NO: 81 - protein, 8 aa, Artificial Sequence
GFTLNYYM

SEQ ID NO: 82 - protein, 8 aa, Artificial Sequence
ISAGDGST

SEQ ID NO: 83 - protein, 19 aa, Artificial Sequence
AAGNEGAITWGFGPYEYDY

SEQ ID NO: 84 - protein, 7 aa, Artificial Sequence
GFTLNYY

SEQ ID NO: 85 - protein, 6 aa, Artificial Sequence
SAGDGS

SEQ ID NO: 86 - protein, 5 aa, Artificial Sequence
YYMMG

SEQ ID NO: 87 - protein, 5 aa, Artificial Sequence
IHIMS

SEQ ID NO: 88 - protein, 16 aa, Artificial Sequence
NIRNDGSTYYVDSVKG

SEQ ID NO: 89 - protein, 16 aa, Artificial Sequence
GIRNDGSTYYVDSVKG

SEQ ID NO: 90 - protein, 16 aa, Artificial Sequence
GIRNDGSTVYVDSVKG

SEQ ID NO: 91 - protein, 16 aa, Artificial Sequence
GIRNDGSTVYADSVKG

SEQ ID NO: 92 - protein, 122 aa, Artificial Sequence
EVQVVESGGGLVQPGGSLRLSCAASGFTFSSSAMSWARQAPGKGLEWVSGIYPDGSAEYTDSMKGRFTITRDNAKNTVYLQMNSLKPEDTAVYYCAIGRGPSIQAMFRPGGWGQGTQVTVSS

SEQ ID NO: 93 - protein, 120 aa, Artificial Sequence
EVQVVESGGGLVQPGGSLRLSCAASGFTFSSSAMSWARQAPGKGREWVSGIYPDGSTEYADSMKGRFTITRDNAQNTVYLQMDNLRPEDTAVYYCAVGRPINADRPSELWGRGTQVTVSS

SEQ ID NO: 94 - protein, 122 aa, Artificial Sequence
QVQLVESGGGLVQPGGSLRLSCAASGSIFSIYAMGWYRQAPGKQRELVAAITSGTNTYYRDSVKGRFTISRDNAKNTVYLQMNSLKPEDTAVYSCNVAPWGDYDGAADFVSWGQGTQVTVSS

SEQ ID NO: 95 - protein, 125 aa, Artificial Sequence
QLQLVESGGGLVQAGGSLRLSCEASGSIFSINAIGWFRQAPGKEREGVSCISRSDGKTYYADSVKGRFTISRDNAKNTVYLQMNSLKPEDTAVYYCATDPSTRYGCYDPALFDSWGQGTQVTVSS

SEQ ID NO: 96 - protein, 122 aa, Artificial Sequence
QVQLVESGGGLVQPGGSLRLSCAASGSISSIYAMGWYRQAPGKQRELVAAIRSAGSTFYRDSVKGRFTISRDNVKNTVYLQMNSLKPEDTAVYQCNVAPWGDYDGAADFTSWGQGTQVTVSS

SEQ ID NO: 97 - protein, 122 aa, Artificial Sequence
EVQVVESGGGLVQPGGSLRLSCAASGSIFNIYAMGWYRQAPGKQRELVAAITSGGSTYYRESVKGRFTISRDNAKNTMYLQMNSLKPEDTAVYYCNVAPWGDYDGAADFDSWGQGTQVTVSS

SEQ ID NO: 98 - protein, 126 aa, Artificial Sequence
QLQLVESGGGLVQPGGSLRLSCAGSGFTLDYYMIGWFRQAPGKEREGLSCISPADGSTYYADSVKGRFTISRDSAKNTVYLQMNSLKPEDTALYYCAAGNEGGISWGFGPYEYDYWGQGTQVTVSS

SEQ ID NO: 99 - protein, 126 aa, Artificial Sequence
QLQLVESGGGLVQPGESLRLSCTGSGFTLAYYMIGWFRQAPGKEREGLSCISPADGSTYYADSVKGRFTISRDNAKNVVYLQMNNLKPEDTGVYYCAAGNEAAITWGFGPYEYDQWGQGTQVTVSS

SEQ ID NO: 100 - protein, 126 aa, Artificial Sequence
QVQLVESGGGLVQPGGSLRLSCTGSGFTLDYYMIGWFRQAPGKEREGLSCISSGDGSTYYADSVKGRFTISRDNAKNTVYLQMNSLKPEDTAVYYCAAGNEATITWGFGPWEYDYWGQGTQVTVSS

SEQ ID NO: 101 - protein, 122 aa, Artificial Sequence
QVQLVESGGRLVQPGESLRLSCVASGFTFSSSAMSWARQAPGKGLEWMSGIYPDGTPVYADSMKGRFTVSRDNAKNMVYLQMNSLKPEDTAVYYCAVGIRLSDYQGQRRQLLGQGTQVTVSS

SEQ ID NO: 102 - protein, 16 aa, Artificial Sequence
GIYPDGSAEYTDSMKG

SEQ ID NO: 103 - protein, 14 aa, Artificial Sequence
GRGPSIQAMFRPGG

SEQ ID NO: 104 - protein, 8 aa, Artificial Sequence
GFTFSSSA

SEQ ID NO: 105 - protein, 7 aa, Artificial Sequence
IYPDGSA

SEQ ID NO: 106 - protein, 16 aa, Artificial Sequence
AIGRGPSIQAMFRPGG

SEQ ID NO: 107 - protein, 7 aa, Artificial Sequence
GFTFSSS

SEQ ID NO: 108 - protein, 5 aa, Artificial Sequence
YPDGS

SEQ ID NO: 109 - protein, 16 aa, Artificial Sequence
GIYPDGSTEYADSMKG

SEQ ID NO: 110 - protein, 12 aa, Artificial Sequence
GRPINADRPSEL

SEQ ID NO: 111 - protein, 7 aa, Artificial Sequence
IYPDGST

SEQ ID NO: 112 - protein, 14 aa, Artificial Sequence
AVGRPINADRPSEL

SEQ ID NO: 113 - protein, 5 aa, Artificial Sequence
IYAMG

SEQ ID NO: 114 - protein, 16 aa, Artificial Sequence
AITSGTNTYYRDSVKG

SEQ ID NO: 115 - protein, 14 aa, Artificial Sequence
APWGDYDGAADFVS

SEQ ID NO: 116 - protein, 8 aa, Artificial Sequence
GSIFSIYA

SEQ ID NO: 117 - protein, 7 aa, Artificial Sequence
ITSGTNT

SEQ ID NO: 118 - protein, 16 aa, Artificial Sequence
NVAPWGDYDGAADFVS

SEQ ID NO: 119 - protein, 7 aa, Artificial Sequence
GSIFSIY

SEQ ID NO: 120 - protein, 5 aa, Artificial Sequence
TSGTN

SEQ ID NO: 121 - protein, 5 aa, Artificial Sequence
INAIG

SEQ ID NO: 122 - protein, 17 aa, Artificial Sequence
CISRSDGKTYYADSVKG

SEQ ID NO: 123 - protein, 16 aa, Artificial Sequence
DPSTRYGCYDPALFDS

SEQ ID NO: 124 - protein, 8 aa, Artificial Sequence
GSIFSINA

SEQ ID NO: 125 - protein, 8 aa, Artificial Sequence
ISRSDGKT

SEQ ID NO: 126 - protein, 18 aa, Artificial Sequence
ATDPSTRYGCYDPALFDS

SEQ ID NO: 127 - protein, 7 aa, Artificial Sequence
GSIFSIN

SEQ ID NO: 128 - protein, 6 aa, Artificial Sequence
SRSDGK

SEQ ID NO: 129 - protein, 16 aa, Artificial Sequence
AIRSAGSTFYRDSVKG

SEQ ID NO: 130 - protein, 14 aa, Artificial Sequence
APWGDYDGAADFTS

SEQ ID NO: 131 - protein, 8 aa, Artificial Sequence
GSISSIYA

SEQ ID NO: 132 - protein, 7 aa, Artificial Sequence
IRSAGST

SEQ ID NO: 133 - protein, 16 aa, Artificial Sequence
NVAPWGDYDGAADFTS

SEQ ID NO: 134 - protein, 7 aa, Artificial Sequence
GSISSIY

SEQ ID NO: 135 - protein, 5 aa, Artificial Sequence
RSAGS

SEQ ID NO: 136 - protein, 16 aa, Artificial Sequence
AITSGGSTYYRESVKG

SEQ ID NO: 137 - protein, 14 aa, Artificial Sequence
APWGDYDGAADFDS

SEQ ID NO: 138 - protein, 8 aa, Artificial Sequence
GSIFNIYA

SEQ ID NO: 139 - protein, 7 aa, Artificial Sequence
ITSGGST

SEQ ID NO: 140 - protein, 16 aa, Artificial Sequence
NVAPWGDYDGAADFDS

SEQ ID NO: 141 - protein, 7 aa, Artificial Sequence
GSIFNIY

SEQ ID NO: 142 - protein, 5 aa, Artificial Sequence
TSGGS

SEQ ID NO: 143 - protein, 17 aa, Artificial Sequence
CISPADGSTYYADSVKG

SEQ ID NO: 144 - protein, 17 aa, Artificial Sequence
GNEGGISWGFGPYEYDY

SEQ ID NO: 145 - protein, 19 aa, Artificial Sequence
AAGNEGGISWGFGPYEYDY

SEQ ID NO: 146 - protein, 17 aa, Artificial Sequence
GNEAAITWGFGPYEYDQ

SEQ ID NO: 147 - protein, 19 aa, Artificial Sequence
AAGNEAAITWGFGPYEYDQ

SEQ ID NO: 148 - protein, 17 aa, Artificial Sequence
CISSGDGSTYYADSVKG

SEQ ID NO: 149 - protein, 17 aa, Artificial Sequence
GNEATITWGFGPWEYDY

SEQ ID NO: 150 - protein, 8 aa, Artificial Sequence
ISSGDGST

SEQ ID NO: 151 - protein, 19 aa, Artificial Sequence
AAGNEATITWGFGPWEYDY

SEQ ID NO: 152 - protein, 6 aa, Artificial Sequence
SSGDGS

SEQ ID NO: 153 - protein, 16 aa, Artificial Sequence
GIYPDGTPVYADSMKG

SEQ ID NO: 154 - protein, 14 aa, Artificial Sequence
GIRLSDYQGQRRQL

SEQ ID NO: 155 - protein, 7 aa, Artificial Sequence
IYPDGTP

SEQ ID NO: 156 - protein, 16 aa, Artificial Sequence
AVGIRLSDYQGQRRQL

SEQ ID NO: 157 - protein, 5 aa, Artificial Sequence
YPDGT